European Patent Specification EP 3 743 113 B1, published April 8, 2026. Title: Expression vector and method. Applicant: Southern Eye Equipment. The sequence listing filed with the application follows.

SEQUENCE LISTING (48 sequences)

SEQ ID NO: 1 - DNA, 1444 bp, Artificial Sequence
  Synthetic
cctgcaggcagctgcgcgctcgctcgctcactgaggccgcccgggcaaagcccgggcgtcgggcgacctttggtcgcccggcctcagtgagcgagcgagcgcgcagagagggagtggccaactccatcactaggggttcctgcggccgcacgcgtataacttcgtatagcatacattatacgaagttatagatctaacttgtttattgcagcttataatggttacaaataaggcaatagcatcacaaatttcacaaataaggcatttttttcactgcattctagttttggtttgtccaaactcatcaatgtatcttatcatgtctggatctactcgagctgcagtctagagaattcacctgcaggccagtaggcgccggtcacagcttggatctgtaacggcgcagaacagaaaacgaaacaaagacgtagagttgagcaagcagggtcaggcaaagcgtggagagccggctgagtctaggtaggctccaagggagcgccggacaaaggcccggtctcgacctgagctttaaacttacctagacggcggacgcagttcaggaggcaccacaggcgggaggcggcagaacgcgactcaaccggcgtggatggcggcctcaggtagggcggcgggcgcgtgaaggagagatgcgagcccctcgaagcttcagctgtgttctggcggcaaacccgttgcgaaaaagaacgttcacggcgactactgcacttatatacggttctcccccaccctcgggaaaaaggcggagccagtacacgacatcactttcccagtttaccccgcgccaccttctctaggcacccgttcaattgccgacccctccccccaacttctcggggactgtgggcgatgtgcgctctgcccactgacgggcaccggagcgatcgcagatccgtggaattatcacctcgagaataaaatatctttattttcattacatctgtgtgttggttttttgtgtgaatcgatagtactaacatacgctctccatcaaaacaaaacgaaacaaaacaaactagcaaaataggctgtccccagtgcaagtgcaggtgccagaacatttctctctcgagttcgaagtcgacgctagctgggatccagacatgataagatacattgatgagtttggacaaaccaaaactagaatgcagtgaaaaaaatgccttatttgtgaaatttgtgatgctattgccttatttgtaaccattataagctgcaataaacaagttataacttcgtatagcatacattatacgaagttatcacgtgcggaccgagcggccgcaggaacccctagtgatggagttggccactccctctctgcgcgctcgctcgctcactgaggccgggcgaccaaaggtcgcccgacgcccgggctttgcccgggcggcctcagtgagcgagcgagcgcgcagctgcctgcagg

SEQ ID NO: 2 - DNA, 747 bp, Artificial Sequence
  Synthetic
atgtctagactggacaagagcaaagtcataaacggagctctggaattactcaatggtgtcggtatcgaaggcctgacgacaaggaaactcgctcaaaagctgggagttgagcagcctaccctgtactggcacgtgaagaacaagcgggccctgctcgatgccctgccaatcgagatgctggacaggcatcatacccacttctgccccctggaaggcgagtcatggcaagactttctgcggaacaacgccaagtcataccgctgtgctctcctctcacatcgcgacggggctaaagtgcatctcggcacccgcccaacagagaaacagtacgaaaccctggaaaatcagctcgcgttcctgtgtcagcaaggcttctccctggagaacgcactgtacgctctgtccgccgtgggccactttacactgggctgcgtattggaggaacaggagcatcaagtagcaaaagaggaaagagagacacctaccaccgattctatgcccccacttctgagacaagcaattgagctgttcgaccggcagggagccgaacctgccttccttttcggcctggaactaatcatatgtggcctggagaaacagctaaagtgcgaaagcggcgggccgaccgacgcccttgacgattttgacttagacatgctcccagccgatgcccttgacgactttgaccttgatatgctgcctgctgacgctcttgacgattttgaccttgacatgctccccgggtaa

SEQ ID NO: 3 - DNA, 617 bp, Artificial Sequence
  Synthetic
atgagtccaaagagaagaacacaggcagagcgcgcaatggagacccagggcaagttgattgcagcggccctgggggttttacgggaaaaaggttacgcgggattccggatcgcagatgtgcccggtgctgcaggtgtctcgagaggagcgcagagccatcatttcccgacaaagcttgagcttctgcttgccacttttgaatggctttacgaacagatcaccgaacgcagtcgggctcgattagcgaaattgaagccagaggatgacgtcatccagcaaatgctggacgacgccgccgaatttttcctcgacgatgacttctctatcagccttgatttgattgtggctgccgaccgggatccagcgttacgcgagggtattcagcgcacggtagagaggaatcggtttgtcgtcgaggatatgtggcttggtgttctggtgagccgtggtctttcgcgtgatgatgcagaagatatcctttggttgatattcaattcggtgcgtgggcttgctgttcgtagcctatggcagaaggacaaagaacgctttgagcgtgtcaggaactcgacactcgaaattgcgcgagagcggtacgcgaaattcaagcgctagtctag

SEQ ID NO: 4 - DNA, 315 bp, Artificial Sequence
  Synthetic
gagtttactccctatcagtgatagagaacgtatgtcgagtttactccctatcagtgatagagaacgatgtcgagtttactccctatcagtgatagagaacgtatgtcgagtttactccctatcagtgatagagaacgtatgtcgagtttactccctatcagtgatagagaacgtatgtcgagtttatccctatcagtgatagagaacgtatgtcgagtttactccctatcagtgatagagaacgtatgtcgaggtaggcgtgtacggtgggaggcctatataagcagagctcgtttagtgaaccgtcagatcgcc

SEQ ID NO: 5 - DNA, 584 bp, Artificial Sequence
  Synthetic
cctaggcgttacataacttacggtaaatggcccgcctggctgaccgcccaacgacccccgcccattgacgtcaataatgacgtatgttcccatagtaacgccaatagggactttccattgacgtcaatgggtggagtatttacggtaaactgcccacttggcagtacatcaagtgtatcatatgccaagtccgccccctattgacgtcaatgacggtaaatggcccgcctggcattatgcccagtacatgaccttacgggactttcctacttggcagtacatctacgtattagtcatcgctattaccatggtgatgcggttttggcagtacaccaatgggcgtggatagcggtttgactcacggggatttccaagtctccaccccattgacgtcaatgggagtttgttttggcaccaaaatcaacgggactttccaaaatgtcgtaataaccccgccccgttgacgcaaatgggcaagcttgccgggtcgaggtaggcgtgtacggtgggaggcctatataagcaaccggtataatacaaacagaccagattgtctgtttgttcaattggaagaaggatcctct

SEQ ID NO: 6 - DNA, 621 bp, Artificial Sequence
  Synthetic
gggtcattagttcatagcccatatatggagttccgcgttacataacttacggtaaatggcccgcctggctgaccgcccaacgacccccgcccattgacgtcaataatgacgtatgttcccatagtaacgtcaatagggactttccattgacgtcaatgggtggagtatttacggtaaactgcccacttggcagtacatcaagtgtatcatatgccaagtacgccccctattgacgtcaatgacggtaaatggcccgcctggcattatgcccagtacatgaccttatgggactttcctacttggcagtacatctacgtattagtcatcgctattaccatggtgatgcggttttggcagtacatcaatgggcgtggatagcggtttgactcacggggatttccaagtctccaccccattgacgtcaatgggagtttgttttgcaccaaaatcaacgggactttccaaaatgtcgtaacaactccgccccattgacgcaaatgggcggtaggcgtgtacggtgggaggtctatataagcagagctcgtttagtgaaccgtcagatcgcctggagacgccatccacgctgttttgacctccatagaagacaccgggaccgatcca

SEQ ID NO: 7 - DNA, 726 bp, Artificial Sequence
  Synthetic
atggtttctaagggagaagaactctttactggtgttgtcccaattctggttgagctggatggtgatgtgaatggccacaaattctctgtgtctggtgaaggtgaaggagatgcaacttatggaaagctgactctgaagttcatttgtacaacaggaaagctgccagtgccttggccaactctggtgaccaccctgacttatggtgttcaatgtttcagcaggtaccctgaccacatgaagcagcatgacttctttaaatctgcaatgccagaaggttatgttcaggagaggacaatcttctttaaggatgatggaaattataagacaagggcagaagtgaagtttgaaggtgatacactggttaacagaattgagctgaaaggcattgattttaaggaagatggaaacattctgggtcacaagctggagtacaactataattctcacaatgtttacattatggcagataagcagaggaatggaattaaggctaatttcaagattagacacaacattgaggatggatctgtccaactggcagaccattaccagcagaacacccctattggtgatggcccagttctcctcccagataatcactatctcagcactcaatctgctctgtccaaagaccctaatgagaaaagagaccacatggtcctcctggagtttgtgacagcagcaggaattactctgggaatggatgagctgtacaagtaaagctag

SEQ ID NO: 8 - DNA, 570 bp, Homo sapiens
atgcacagctcagcactgctctgttgcctggtcctcctgactggggtgagggccagcccaggccagggcacccagtctgagaacagctgcacccacttcccaggcaacctgcctaacatgcttcgagatctccgagatgccttcagcagagtgaagactttctttcaaatgaaggatcagctggacaacttgttgttaaaggagtccttgctggaggactttaagggttacctgggttgccaagccttgtctgagatgatccagttttacctggaggaggtgatgccccaagctgagaaccaagacccagacatcaaggcgcatgtgaactccctgggggagaacctgaagaccctcaggctgaggctacggcgctgtcatcgatttcttccctgtgaaaacaagagcaaggccgtggagcaggtgaagaatgcctttaataagctccaagagaaaggcatctacaaagccatgagtgagtttgacatcttcatcaactacatagaagcctacatgacaatgaagatacgaaactgagacatcagggtggcgactctatagactcgctag

SEQ ID NO: 9 - DNA, 1739 bp, Artificial Sequence
  Synthetic
atgtacagaatgcagctgctgagctgtatcgccctgtctctggccctggtcacaaactctgcccacagccacagagacttccagcctgtgctgcatctggtggccctgaactctccactgtctggcggcatgagaggcatcagaggcgccgacttccagtgtttccagcaggctagagctgtcggcctggccggaacattcagagcctttctgagcagcagactgcaggacctgtacagcatcgtgcggagagccgatagagccgctgtgcctatcgtgaacctgaaggacgagctgctgttccctagctgggaagctctgttctctggcagcgagggacctctgaaaccaggcgccagaatcttcagcttcgacggcaaggacgtgctgagacaccctacctggcctcagaaatctgtgtggcacggcagcgatcccaacggcagaaggctgacagagagctactgcgagacttggaggacagaggcccctagcgctacaggccaagcaagctcacttctcggaggcagactgctgggacagtctgccgcttcttgtcaccacgcctacatcgtgctgtgcatcgagaacagcttcatgaccgccagcaaggtgccaggcgtgggaacaaatagcgtgtacctgagcgagtgcaagaccggcaacggcaagaactacagaggcaccatgagcaagaccaagaacggcatcacctgtcagaagtggtccagcacaagccctcacagacccagattcagccctgctacacacccaagcgaaggcctggaagagaactactgcagaaaccccgacaacgaccctcaaggcccttggtgctacaccaccgatcctgagaagagatacgactactgcgacatcctggaatgcgaagaggaatgcatgcactgcagcggcgagaactacgatggcaagatctccaagaccatgagcggcctcgagtgtcaggcctgggattctcagtctcctcacgctcacggctacatccccagcaagttccccaacaagaatctgaagaagaattactgtcggaaccccgaccgcgagctgaggccttggtgtttcacaacagaccctaacaagagatgggagctgtgtgacatccctagatgcaccacacctccaccttctagcggccctacctaccagtgtctgaaaggcaccggcgagaattacaggggcaatgtggccgtgaccgtgtctggacacacatgccaacattggagcgcccagacacctcacacacacaacagaacccctgagaacttcccctgcaagaacctggacgaaaactattgccggaatcctgacggcaagagggccccttggtgtcacactaccaacagccaagtccgctgggagtactgcaagatccccagctgtgacagcagccctgtgtctacagaacagctggcccctacagctcctcctgagctgacacctgtggtgcaggactgttatcacggcgacggccagtcctacagaggaacaagcagcaccaccacaaccggcaagaagtgccagagctggtctagcatgacccctcacaggcaccagaaaaccccagagaattaccccaacgccggcctgaccatgaactactgtaggaatccagacgccgacaaaggcccctggtgttttaccacagatcccagcgtcagatgggaatactgtaacctgaagaagtgcagcggcaccgaggccagcgttgtgtgagctag

SEQ ID NO: 10 - DNA, 542 bp, Homo sapiens
atggaaatctgcaggggaccttacagtcacctaatctctctccttctcatccttctgtttcgttcagagtcagctggccaccctgctgggaaaagaccctgcaagatgcaagccttcagaatctgggatactaaccagaagaccttctacctgaggaacaaccagctcattgctgggtacttacaaggaccaaataccaaactagaagaaaagatagacatggtgcctattgactttcggaatgtgttcttgggcatccacgggggcaagctgtgcctgtcttgtgtcaagtctggagatgacaccaagctccagctggaggaggttaacatcactgatctgaacaagaacaaagaagaagacaagcgctttaccttcatccgctccgagacaggccctaccaccagcttcgaatcacttgcctgtccaggatggttcctctgcacaacactagaggctgatcatcccgtgagcctcaccaacacaccaaaagagccctgtacagtcacaaagttctacttccaggaagaccaataggctag

SEQ ID NO: 11 - DNA, 2315 bp, Artificial Sequence
  Synthetic
atgcacagctcagcactgctctgttgcctggtcctcctgactggggtgagggccagcccaggccagggcacccagtctgagaacagctgcacccacttcccaggcaacctgcctaacatgcttcgagatctccgagatgccttcagcagagtgaagactttctttcaaatgaaggatcagctggacaacttgttgttaaaggagtccttgctggaggactttaagggttacctgggttgccaagccttgtctgagatgatccagttttacctggaggaggtgatgccccaagctgagaaccaagacccagacatcaaggcgcatgtgaactccctgggggagaacctgaagaccctcaggctgaggctacggcgctgtcatcgatttcttccctgtgaaaacaagagcaaggccgtggagcaggtgaagaatgcctttaataagctccaagagaaaggcatctacaaagccatgagtgagtttgacatcttcatcaactacatagaagcctacatgacaatgaagatacgaaacggaagcggagctactaacttcagcctgctgaagcaggctggcgacgtggaggagaaccctggacctggtctccggccgatggaaatctgcagaggcctccgcagtcacctaatcactctcctcctcttcctgttccattcagagacgatctgccgaccctctgggagaaaatccagcaagatgcaagccttcagaatctgggatgttaaccagaagaccttctatctgaggaacaaccaactagttgccggatacttgcaaggaccaaatgtcaatttagaagaaaagatagatgtggtacccattgagcctcatgctctgttcttgggaatccatggagggaagatgtgcctgtcctgtgtcaagtctggtgatgagaccagactccagctggaggcagttaacatcactgacctgagcgagaacagaaagcaggacaagcgcttcgccttcatccgctcagacagtggccccaccaccagttttgagtctgccgcctgccccggttggttcctctgcacagcgatggaagctgaccagcccgtcagcctcaccaatatgcctgacgaaggcgtcatggtcaccaaattctacttccaggaggacgagtaggctagcgtcgacgccaccatgcacagctcagcactgctctgttgcctggtcctcctgactggggtgagggccagcccaggccagggcacccagtctgagaacagctgcacccacttcccaggcaacctgcctaacatgcttcgagatctccgagatgccttcagcagagtgaagactttctttcaaatgaaggatcagctggacaacttgttgttaaaggagtccttgctggaggactttaagggttacctgggttgccaagccttgtctgagatgatccagttttacctggaggaggtgatgccccaagctgagaaccaagacccagacatcaaggcgcatgtgaactccctgggggagaacctgaagaccctcaggctgaggctacggcgctgtcatcgatttcttccctgtgaaaacaagagcaaggccgtggagcaggtgaagaatgcctttaataagctccaagagaaaggcatctacaaagccatgagtgagtttgacatcttcatcaactacatagaagcctacatgacaatgaagatacgaaacggaagcggagctactaacttcagcctgctgaagcaggctggcgacgtggaggagaaccctggacctggtctccggccgatggaaatctgcagaggcctccgcagtcacctaatcactctcctcctcttcctgttccattcagagacgatctgccgaccctctgggagaaaatccagcaagatgcaagccttcagaatctgggatgttaaccagaagaccttctatctgaggaacaaccaactagttgccggatacttgcaaggaccaaatgtcaatttagaagaaaagatagatgtggtacccattgagcctcatgctctgttcttgggaatccatggagggaagatgtgcctgtcctgtgtcaagtctggtgatgagaccagactccagctggaggcagttaacatcactgacctgagcgagaacagaaagcaggacaagcgcttcgccttcatccgctcagacagtggccccaccaccagttttgagtctgccgcctgccccggttggttcctctgcacagcgatggaagctgaccagcccgtcagcctcaccaatatgcctgacgaaggcgtcatggtcaccaaattctacttccaggaggacgagtaggctag

SEQ ID NO: 12 - DNA, 614 bp, Artificial Sequence
  Synthetic
atgaactccttctccacaagcgccttcggtccagttgccttctccctgggcctgctcctggtgttgcctgctgccttccctgccccagtcttcacactcgaagatttcgttggggactggcgacagacagccggctacaacctggaccaagtccttgaacagggaggtgtgtccagtttgtttcagaatctcggggtgtccgtaactccgatccaaaggattgtcctgagcggtgaaaatgggctgaagatcgacatccatgtcatcatcccgtatgaaggtctgagcggcgaccaaatgggccagatcgaaaaaatttttaaggtggtgtaccctgtggatgatcatcactttaaggtgatcctgcactatggcacactggtaatcgacggggttacgccgaacatgatcgactatttcggacggccgtatgaaggcatcgccgtgttcgacggcaaaaagatcactgtaacagggaccctgtggaacggcaacaaaattatcgacgagcgcctgatcaaccccgacggctccctgctgttccgagtaaccatcaacggagtgaccggctggcggctgtgcgaacgcattctggcgtaaggccgcgactctag

SEQ ID NO: 13 - DNA, 34 bp, Artificial Sequence
  Synthetic
ataacttcgtatagcatacattatacgaagttat

SEQ ID NO: 14 - DNA, 179 bp, Artificial Sequence
  Synthetic
gtggaattatcacctcgagaataaaatatctttattttcattacatctgtgtgttggttttttgtgtgaatcgatagtactaacatacgctctccatcaaaacaaaacgaaacaaaacaaactagcaaaataggctgtccccagtgcaagtgcaggtgccagaacatttctctctcgag

SEQ ID NO: 15 - DNA, 6977 bp, Artificial Sequence
  Synthetic sequence
cctgcaggcagctgcgcgctcgctcgctcactgaggccgcccgggcaaagcccgggcgtcgggcgacctttggtcgcccggcctcagtgagcgagcgagcgcgcagagagggagtggccaactccatcactaggggttcctgcggccgcacgcgtataacttcgtatagcatacattatacgaagttatagatctaacttgtttattgcagcttataatggttacaaataaggcaatagcatcacaaatttcacaaataaggcatttttttcactgcattctagttttggtttgtccaaactcatcaatgtatcttatcatgtctggatctactcgagctgcagtctagactagcgcttgaatttcgcgtaccgctctcgcgcaatttcgagtgtcgagttcctgacacgctcaaagcgttctttgtccttctgccataggctacgaacagcaagcccacgcaccgaattgaatatcaaccaaaggatatcttctgcatcatcacgcgaaagaccacggctcaccagaacaccaagccacatatcctcgacgacaaaccgattcctctctaccgtgcgctgaataccctcgcgtaacgctggatcccggtcggcagccacaatcaaatcaaggctgatagagaagtcatcgtcgaggaaaaattcggcggcgtcgtccagcatttgctggatgacgtcatcctctggcttcaatttcgctaatcgagcccgactgcgttcggtgatctgttcgtaaagccattcaaaagtggcaagcagaagctcaagctttgtcgggaaatgatggctctgcgctcctctcgagacacctgcagcaccgggcacatctgcgatccggaatcccgcgtaacctttttcccgtaaaacccccagggccgctgcaatcaacttgccctgggtctccattgcgcgctctgcctgtgttcttctctttggactcatgaattcacctgcaggccagtaggcgccggtcacagcttggatctgtaacggcgcagaacagaaaacgaaacaaagacgtagagttgagcaagcagggtcaggcaaagcgtggagagccggctgagtctaggtaggctccaagggagcgccggacaaaggcccggtctcgacctgagctttaaacttacctagacggcggacgcagttcaggaggcaccacaggcgggaggcggcagaacgcgactcaaccggcgtggatggcggcctcaggtagggcggcgggcgcgtgaaggagagatgcgagcccctcgaagcttcagctgtgttctggcggcaaacccgttgcgaaaaagaacgttcacggcgactactgcacttatatacggttctcccccaccctcgggaaaaaggcggagccagtacacgacatcactttcccagtttaccccgcgccaccttctctaggcacccgttcaattgccgacccctccccccaacttctcggggactgtgggcgatgtgcgctctgcccactgacgggcaccggagcgatcgcagatccgtggaattatcacctcgagaataaaatatctttattttcattacatctgtgtgttggttttttgtgtgaatcgatagtactaacatacgctctccatcaaaacaaaacgaaacaaaacaaactagcaaaataggctgtccccagtgcaagtgcaggtgccagaacatttctctctcgagttcgaacctaggcgttacataacttacggtaaatggcccgcctggctgaccgcccaacgacccccgcccattgacgtcaataatgacgtatgttcccatagtaacgccaatagggactttccattgacgtcaatgggtggagtatttacggtaaactgcccacttggcagtacatcaagtgtatcatatgccaagtccgccccctattgacgtcaatgacggtaaatggcccgcctggcattatgcccagtacatgaccttacgggactttcctacttggcagtacatctacgtattagtcatcgctattaccatggtgatgcggttttggcagtacaccaatgggcgtggatagcggtttgactcacggggatttccaagtctccaccccattgacgtcaatgggagtttgttttggcaccaaaatcaacgggactttccaaaatgtcgtaataaccccgccccgttgacgcaaatgggcaagcttgccgggtcgaggtaggcgtgtacggtgggaggcctatataagcaaccggtataatacaaacagaccagattgtctgtttgttcaattggaagaaggatcctctgtcgacgccaccatgtacagaatgcagctgctgagctgtatcgccctgtctctggccctggtcacaaactctgcccacagccacagagacttccagcctgtgctgcatctggtggccctgaactctccactgtctggcggcatgagaggcatcagaggcgccgacttccagtgtttccagcaggctagagctgtcggcctggccggaacattcagagcctttctgagcagcagactgcaggacctgtacagcatcgtgcggagagccgatagagccgctgtgcctatcgtgaacctgaaggacgagctgctgttccctagctgggaagctctgttctctggcagcgagggacctctgaaaccaggcgccagaatcttcagcttcgacggcaaggacgtgctgagacaccctacctggcctcagaaatctgtgtggcacggcagcgatcccaacggcagaaggctgacagagagctactgcgagacttggaggacagaggcccctagcgctacaggccaagcaagctcacttctcggaggcagactgctgggacagtctgccgcttcttgtcaccacgcctacatcgtgctgtgcatcgagaacagcttcatgaccgccagcaaggtgccaggcgtgggaacaaatagcgtgtacctgagcgagtgcaagaccggcaacggcaagaactacagaggcaccatgagcaagaccaagaacggcatcacctgtcagaagtggtccagcacaagccctcacagacccagattcagccctgctacacacccaagcgaaggcctggaagagaactactgcagaaaccccgacaacgaccctcaaggcccttggtgctacaccaccgatcctgagaagagatacgactactgcgacatcctggaatgcgaagaggaatgcatgcactgcagcggcgagaactacgatggcaagatctccaagaccatgagcggcctcgagtgtcaggcctgggattctcagtctcctcacgctcacggctacatccccagcaagttccccaacaagaatctgaagaagaattactgtcggaaccccgaccgcgagctgaggccttggtgtttcacaacagaccctaacaagagatgggagctgtgtgacatccctagatgcaccacacctccaccttctagcggccctacctaccagtgtctgaaaggcaccggcgagaattacaggggcaatgtggccgtgaccgtgtctggacacacatgccaacattggagcgcccagacacctcacacacacaacagaacccctgagaacttcccctgcaagaacctggacgaaaactattgccggaatcctgacggcaagagggccccttggtgtcacactaccaacagccaagtccgctgggagtactgcaagatccccagctgtgacagcagccctgtgtctacagaacagctggcccctacagctcctcctgagctgacacctgtggtgcaggactgttatcacggcgacggccagtcctacagaggaacaagcagcaccaccacaaccggcaagaagtgccagagctggtctagcatgacccctcacaggcaccagaaaaccccagagaattaccccaacgccggcctgaccatgaactactgtaggaatccagacgccgacaaaggcccctggtgttttaccacagatcccagcgtcagatgggaatactgtaacctgaagaagtgcagcggcaccgaggccagcgttgtgtgagctagctgggatccagacatgataagatacattgatgagtttggacaaaccaaaactagaatgcagtgaaaaaaatgccttatttgtgaaatttgtgatgctattgccttatttgtaaccattataagctgcaataaacaagttataacttcgtatagcatacattatacgaagttatcacgtgcggaccgagcggccgcaggaacccctagtgatggagttggccactccctctctgcgcgctcgctcgctcactgaggccgggcgaccaaaggtcgcccgacgcccgggctttgcccgggcggcctcagtgagcgagcgagcgcgcagctgcctgcaggggcgcctgatgcggtattttctccttacgcatctgtgcggtatttcacaccgcatacgtcaaagcaaccatagtacgcgccctgtagcggcgcattaagcgcggcgggtgtggtggttacgcgcagcgtgaccgctacacttgccagcgccctagcgcccgctcctttcgctttcttcccttcctttctcgccacgttcgccggctttccccgtcaagctctaaatcgggggctccctttagggttccgatttagtgctttacggcacctcgaccccaaaaaacttgatttgggtgatggttcacgtagtgggccatcgccctgatagacggtttttcgccctttgacgttggagtccacgttctttaatagtggactcttgttccaaactggaacaacactcaaccctatctcgggctattcttttgatttataagggattttgccgatttcggcctattggttaaaaaatgagctgatttaacaaaaatttaacgcgaattttaacaaaatattaacgtttacaattttatggtgcactctcagtacaatctgctctgatgccgcatagttaagccagccccgacacccgccaacacccgctgacgcgccctgacgggcttgtctgctcccggcatccgcttacagacaagctgtgaccgtctccgggagctgcatgtgtcagaggttttcaccgtcatcaccgaaacgcgcgagacgaaagggcctcgtgatacgcctatttttataggttaatgtcatgataataatggtttcttagacgtcaggtggcacttttcggggaaatgtgcgcggaacccctatttgtttatttttctaaatacattcaaatatgtatccgctcatgagacaataaccctgataaatgcttcaataatattgaaaaaggaagagtatgagtattcaacatttccgtgtcgcccttattcccttttttgcggcattttgccttcctgtttttgctcacccagaaacgctggtgaaagtaaaagatgctgaagatcagttgggtgcacgagtgggttacatcgaactggatctcaacagcggtaagatccttgagagttttcgccccgaagaacgttttccaatgatgagcacttttaaagttctgctatgtggcgcggtattatcccgtattgacgccgggcaagagcaactcggtcgccgcatacactattctcagaatgacttggttgagtactcaccagtcacagaaaagcatcttacggatggcatgacagtaagagaattatgcagtgctgccataaccatgagtgataacactgcggccaacttacttctgacaacgatcggaggaccgaaggagctaaccgcttttttgcacaacatgggggatcatgtaactcgccttgatcgttgggaaccggagctgaatgaagccataccaaacgacgagcgtgacaccacgatgcctgtagcaatggcaacaacgttgcgcaaactattaactggcgaactacttactctagcttcccggcaacaattaatagactggatggaggcggataaagttgcaggaccacttctgcgctcggcccttccggctggctggtttattgctgataaatctggagccggtgagcgtgggtctcgcggtatcattgcagcactggggccagatggtaagccctcccgtatcgtagttatctacacgacggggagtcaggcaactatggatgaacgaaatagacagatcgctgagataggtgcctcactgattaagcattggtaactgtcagaccaagtttactcatatatactttagattgatttaaaacttcatttttaatttaaaaggatctaggtgaagatcctttttgataatctcatgaccaaaatcccttaacgtgagttttcgttccactgagcgtcagaccccgtagaaaagatcaaaggatcttcttgagatcctttttttctgcgcgtaatctgctgcttgcaaacaaaaaaaccaccgctaccagcggtggtttgtttgccggatcaagagctaccaactctttttccgaaggtaactggcttcagcagagcgcagataccaaatactgtccttctagtgtagccgtagttaggccaccacttcaagaactctgtagcaccgcctacatacctcgctctgctaatcctgttaccagtggctgctgccagtggcgataagtcgtgtcttaccgggttggactcaagacgatagttaccggataaggcgcagcggtcgggctgaacggggggttcgtgcacacagcccagcttggagcgaacgacctacaccgaactgagatacctacagcgtgagctatgagaaagcgccacgcttcccgaagggagaaaggcggacaggtatccggtaagcggcagggtcggaacaggagagcgcacgagggagcttccagggggaaacgcctggtatctttatagtcctgtcgggtttcgccacctctgacttgagcgtcgatttttgtgatgctcgtcaggggggcggagcctatggaaaaacgccagcaacgcggcctttttacggttcctggccttttgctggccttttgctcacatgt

SEQ ID NO: 16 - DNA, 5819 bp, Artificial Sequence
  Synthetic
cctgcaggcagctgcgcgctcgctcgctcactgaggccgcccgggcaaagcccgggcgtcgggcgacctttggtcgcccggcctcagtgagcgagcgagcgcgcagagagggagtggccaactccatcactaggggttcctgcggccgcacgcgtataacttcgtatagcatacattatacgaagttatagatctaacttgtttattgcagcttataatggttacaaataaggcaatagcatcacaaatttcacaaataaggcatttttttcactgcattctagttttggtttgtccaaactcatcaatgtatcttatcatgtctggatctactcgagctgcagtctagactagcgcttgaatttcgcgtaccgctctcgcgcaatttcgagtgtcgagttcctgacacgctcaaagcgttctttgtccttctgccataggctacgaacagcaagcccacgcaccgaattgaatatcaaccaaaggatatcttctgcatcatcacgcgaaagaccacggctcaccagaacaccaagccacatatcctcgacgacaaaccgattcctctctaccgtgcgctgaataccctcgcgtaacgctggatcccggtcggcagccacaatcaaatcaaggctgatagagaagtcatcgtcgaggaaaaattcggcggcgtcgtccagcatttgctggatgacgtcatcctctggcttcaatttcgctaatcgagcccgactgcgttcggtgatctgttcgtaaagccattcaaaagtggcaagcagaagctcaagctttgtcgggaaatgatggctctgcgctcctctcgagacacctgcagcaccgggcacatctgcgatccggaatcccgcgtaacctttttcccgtaaaacccccagggccgctgcaatcaacttgccctgggtctccattgcgcgctctgcctgtgttcttctctttggactcatgaattcacctgcaggccagtaggcgccggtcacagcttggatctgtaacggcgcagaacagaaaacgaaacaaagacgtagagttgagcaagcagggtcaggcaaagcgtggagagccggctgagtctaggtaggctccaagggagcgccggacaaaggcccggtctcgacctgagctttaaacttacctagacggcggacgcagttcaggaggcaccacaggcgggaggcggcagaacgcgactcaaccggcgtggatggcggcctcaggtagggcggcgggcgcgtgaaggagagatgcgagcccctcgaagcttcagctgtgttctggcggcaaacccgttgcgaaaaagaacgttcacggcgactactgcacttatatacggttctcccccaccctcgggaaaaaggcggagccagtacacgacatcactttcccagtttaccccgcgccaccttctctaggcacccgttcaattgccgacccctccccccaacttctcggggactgtgggcgatgtgcgctctgcccactgacgggcaccggagcgatcgcagatccgtggaattatcacctcgagaataaaatatctttattttcattacatctgtgtgttggttttttgtgtgaatcgatagtactaacatacgctctccatcaaaacaaaacgaaacaaaacaaactagcaaaataggctgtccccagtgcaagtgcaggtgccagaacatttctctctcgagttcgaacctaggcgttacataacttacggtaaatggcccgcctggctgaccgcccaacgacccccgcccattgacgtcaataatgacgtatgttcccatagtaacgccaatagggactttccattgacgtcaatgggtggagtatttacggtaaactgcccacttggcagtacatcaagtgtatcatatgccaagtccgccccctattgacgtcaatgacggtaaatggcccgcctggcattatgcccagtacatgaccttacgggactttcctacttggcagtacatctacgtattagtcatcgctattaccatggtgatgcggttttggcagtacaccaatgggcgtggatagcggtttgactcacggggatttccaagtctccaccccattgacgtcaatgggagtttgttttggcaccaaaatcaacgggactttccaaaatgtcgtaataaccccgccccgttgacgcaaatgggcaagcttgccgggtcgaggtaggcgtgtacggtgggaggcctatataagcaaccggtataatacaaacagaccagattgtctgtttgttcaattggaagaaggatcctctgtcgacctgagatcaccggtagcatgcacagctcagcactgctctgttgcctggtcctcctgactggggtgagggccagcccaggccagggcacccagtctgagaacagctgcacccacttcccaggcaacctgcctaacatgcttcgagatctccgagatgccttcagcagagtgaagactttctttcaaatgaaggatcagctggacaacttgttgttaaaggagtccttgctggaggactttaagggttacctgggttgccaagccttgtctgagatgatccagttttacctggaggaggtgatgccccaagctgagaaccaagacccagacatcaaggcgcatgtgaactccctgggggagaacctgaagaccctcaggctgaggctacggcgctgtcatcgatttcttccctgtgaaaacaagagcaaggccgtggagcaggtgaagaatgcctttaataagctccaagagaaaggcatctacaaagccatgagtgagtttgacatcttcatcaactacatagaagcctacatgacaatgaagatacgaaactgagacatcagggtggcgactctatagactcgctagctgggatccagacatgataagatacattgatgagtttggacaaaccaaaactagaatgcagtgaaaaaaatgccttatttgtgaaatttgtgatgctattgccttatttgtaaccattataagctgcaataaacaagttataacttcgtatagcatacattatacgaagttatcacgtgcggaccgagcggccgcaggaacccctagtgatggagttggccactccctctctgcgcgctcgctcgctcactgaggccgggcgaccaaaggtcgcccgacgcccgggctttgcccgggcggcctcagtgagcgagcgagcgcgcagctgcctgcaggggcgcctgatgcggtattttctccttacgcatctgtgcggtatttcacaccgcatacgtcaaagcaaccatagtacgcgccctgtagcggcgcattaagcgcggcgggtgtggtggttacgcgcagcgtgaccgctacacttgccagcgccctagcgcccgctcctttcgctttcttcccttcctttctcgccacgttcgccggctttccccgtcaagctctaaatcgggggctccctttagggttccgatttagtgctttacggcacctcgaccccaaaaaacttgatttgggtgatggttcacgtagtgggccatcgccctgatagacggtttttcgccctttgacgttggagtccacgttctttaatagtggactcttgttccaaactggaacaacactcaaccctatctcgggctattcttttgatttataagggattttgccgatttcggcctattggttaaaaaatgagctgatttaacaaaaatttaacgcgaattttaacaaaatattaacgtttacaattttatggtgcactctcagtacaatctgctctgatgccgcatagttaagccagccccgacacccgccaacacccgctgacgcgccctgacgggcttgtctgctcccggcatccgcttacagacaagctgtgaccgtctccgggagctgcatgtgtcagaggttttcaccgtcatcaccgaaacgcgcgagacgaaagggcctcgtgatacgcctatttttataggttaatgtcatgataataatggtttcttagacgtcaggtggcacttttcggggaaatgtgcgcggaacccctatttgtttatttttctaaatacattcaaatatgtatccgctcatgagacaataaccctgataaatgcttcaataatattgaaaaaggaagagtatgagtattcaacatttccgtgtcgcccttattcccttttttgcggcattttgccttcctgtttttgctcacccagaaacgctggtgaaagtaaaagatgctgaagatcagttgggtgcacgagtgggttacatcgaactggatctcaacagcggtaagatccttgagagttttcgccccgaagaacgttttccaatgatgagcacttttaaagttctgctatgtggcgcggtattatcccgtattgacgccgggcaagagcaactcggtcgccgcatacactattctcagaatgacttggttgagtactcaccagtcacagaaaagcatcttacggatggcatgacagtaagagaattatgcagtgctgccataaccatgagtgataacactgcggccaacttacttctgacaacgatcggaggaccgaaggagctaaccgcttttttgcacaacatgggggatcatgtaactcgccttgatcgttgggaaccggagctgaatgaagccataccaaacgacgagcgtgacaccacgatgcctgtagcaatggcaacaacgttgcgcaaactattaactggcgaactacttactctagcttcccggcaacaattaatagactggatggaggcggataaagttgcaggaccacttctgcgctcggcccttccggctggctggtttattgctgataaatctggagccggtgagcgtgggtctcgcggtatcattgcagcactggggccagatggtaagccctcccgtatcgtagttatctacacgacggggagtcaggcaactatggatgaacgaaatagacagatcgctgagataggtgcctcactgattaagcattggtaactgtcagaccaagtttactcatatatactttagattgatttaaaacttcatttttaatttaaaaggatctaggtgaagatcctttttgataatctcatgaccaaaatcccttaacgtgagttttcgttccactgagcgtcagaccccgtagaaaagatcaaaggatcttcttgagatcctttttttctgcgcgtaatctgctgcttgcaaacaaaaaaaccaccgctaccagcggtggtttgtttgccggatcaagagctaccaactctttttccgaaggtaactggcttcagcagagcgcagataccaaatactgtccttctagtgtagccgtagttaggccaccacttcaagaactctgtagcaccgcctacatacctcgctctgctaatcctgttaccagtggctgctgccagtggcgataagtcgtgtcttaccgggttggactcaagacgatagttaccggataaggcgcagcggtcgggctgaacggggggttcgtgcacacagcccagcttggagcgaacgacctacaccgaactgagatacctacagcgtgagctatgagaaagcgccacgcttcccgaagggagaaaggcggacaggtatccggtaagcggcagggtcggaacaggagagcgcacgagggagcttccagggggaaacgcctggtatctttatagtcctgtcgggtttcgccacctctgacttgagcgtcgatttttgtgatgctcgtcaggggggcggagcctatggaaaaacgccagcaacgcggcctttttacggttcctggccttttgctggccttttgctcacatgt

SEQ ID NO: 17 - protein, 248 aa, Artificial Sequence
  Synthetic
MSRLDKSKVINGALELLNGVGIEGLTTRKLAQKLGVEQPTLYWHVKNKRALLDALPIEMLDRHHTHFCPLEGESWQDFLRNNAKSYRCALLSHRDGAKVHLGTRPTEKQYETLENQLAFLCQQGFSLENALYALSAVGHFTLGCVLEEQEHQVAKEERETPTTDSMPPLLRQAIELFDRQGAEPAFLFGLELIICGLEKQLKCESGGPTDALDDFDLDMLPADALDDFDLDMLPADALDDFDLDMLPG

SEQ ID NO: 18 - protein, 203 aa, Artificial Sequence
  Synthetic
MSPKRRTQAERAMETQGKLIAAALGVLREKGYAGFRIADVPGAAGVSRGAQSHHFPTKLELLLATFEWLYEQITERSRARLAKLKPEDDVIQQMLDDAAEFFLDDDFSISLDLIVAADRDPALREGIQRTVERNRFVVEDMWLGVLVSRGLSRDDAEDILWLIFNSVRGLAVRSLWQKDKERFERVRNSTLEIARERYAKFKR

SEQ ID NO: 19 - protein, 178 aa, Homo sapiens
MHSSALLCCLVLLTGVRASPGQGTQSENSCTHFPGNLPNMLRDLRDAFSRVKTFFQMKDQLDNLLLKESLLEDFKGYLGCQALSEMIQFYLEEVMPQAENQDPDIKAHVNSLGENLKTLRLRLRRCHRFLPCENKSKAVEQVKNAFNKLQEKGIYKAMSEFDIFINYIEAYMTMKIRN

SEQ ID NO: 20 - protein, 577 aa, Artificial Sequence
  Synthetic
MYRMQLLSCIALSLALVTNSAHSHRDFQPVLHLVALNSPLSGGMRGIRGADFQCFQQARAVGLAGTFRAFLSSRLQDLYSIVRRADRAAVPIVNLKDELLFPSWEALFSGSEGPLKPGARIFSFDGKDVLRHPTWPQKSVWHGSDPNGRRLTESYCETWRTEAPSATGQASSLLGGRLLGQSAASCHHAYIVLCIENSFMTASKVPGVGTNSVYLSECKTGNGKNYRGTMSKTKNGITCQKWSSTSPHRPRFSPATHPSEGLEENYCRNPDNDPQGPWCYTTDPEKRYDYCDILECEEECMHCSGENYDGKISKTMSGLECQAWDSQSPHAHGYIPSKFPNKNLKKNYCRNPDRELRPWCFTTDPNKRWELCDIPRCTTPPPSSGPTYQCLKGTGENYRGNVAVTVSGHTCQHWSAQTPHTHNRTPENFPCKNLDENYCRNPDGKRAPWCHTTNSQVRWEYCKIPSCDSSPVSTEQLAPTAPPELTPVVQDCYHGDGQSYRGTSSTTTTGKKCQSWSSMTPHRHQKTPENYPNAGLTMNYCRNPDADKGPWCFTTDPSVRWEYCNLKKCSGTEASVV

SEQ ID NO: 21 - protein, 177 aa, Homo sapiens
MEICRGLRSHLITLLLFLFHSETICRPSGRKSSKMQAFRIWDVNQKTFYLRNNQLVAGYLQGPNVNLEEKIDVVPIEPHALFLGIHGGKMCLSCVKSGDETRLQLEAVNITDLSENRKQDKRFAFIRSDSGPTTSFESAACPGWFLCTAMEADQPVSLTNMPDEGVMVTKFYFQEDE

SEQ ID NO: 22 - DNA, 34 bp, Artificial Sequence; identical to SEQ ID NO: 13
  LoxP site

SEQ ID NO: 23 - DNA, 34 bp, Artificial Sequence
  LoxP site
ataacttcgtataatgtatactatacgaagttat

SEQ ID NO: 24 - DNA, 34 bp, Artificial Sequence
  LoxP site
ataacttcgtataatgtgtactatacgaagttat

SEQ ID NO: 25 - DNA, 34 bp, Artificial Sequence
  LoxP site
ataacttcgtataaagtatcctatacgaagttat

SEQ ID NO: 26 - DNA, 34 bp, Artificial Sequence
  LoxP site
ataacttcgtataagaaaccatatacgaagttat

SEQ ID NO: 27 - DNA, 34 bp, Artificial Sequence
  LoxP site
ataacttcgtatataataccatatacgaagttat

SEQ ID NO: 28 - DNA, 34 bp, Artificial Sequence
  LoxP site
ataacttcgtataagatagaatatacgaagttat

SEQ ID NO: 29 - DNA, 34 bp, Artificial Sequence; identical to SEQ ID NO: 28
  LoxP site

SEQ ID NO: 30 - DNA, 34 bp, Artificial Sequence
  LoxP site
  misc_feature (14)..(16): n is a, c, g, or t
  misc_feature (19)..(21): n is a, c, g, or t
taccgttcgtatannntannntatacgaagttat

SEQ ID NO: 31 - DNA, 34 bp, Artificial Sequence
  LoxP site
  misc_feature (14)..(16): n is a, c, g, or t
  misc_feature (19)..(21): n is a, c, g, or t
ataacttcgtatannntannntatacgaacggta

SEQ ID NO: 32 - DNA, 34 bp, Artificial Sequence
  FRT site
gaagttcctattctctagaaagtataggaacttc

SEQ ID NO: 33 - DNA, 34 bp, Artificial Sequence
  FRT site
gaagttcctatactttctagagaataggaacttc

SEQ ID NO: 34 - DNA, 34 bp, Artificial Sequence
  FRT site
agtgatttgatacttacatgagtaaaggaattag

SEQ ID NO: 35 - DNA, 34 bp, Artificial Sequence
  FRT site
gaagttcctatacttacatgagtaaaggaattag

SEQ ID NO: 36 - DNA, 32 bp, Artificial Sequence
  rox site
taactttaaataatgccaattatttaaagtta

SEQ ID NO: 37 - DNA, 32 bp, Artificial Sequence
  rox site
taactttaaataaggccagttatttaaagtta

SEQ ID NO: 38 - DNA, 32 bp, Artificial Sequence
  rox site
taactttaaataacgcctcttatttaaagtta

SEQ ID NO: 39 - DNA, 32 bp, Artificial Sequence
  rox site
taactttaaataaggcctgttatttaaagtta

SEQ ID NO: 40 - DNA, 32 bp, Artificial Sequence
  rox site
taactttaaataaggcccgttatttaaagtta

SEQ ID NO: 41 - DNA, 32 bp, Artificial Sequence
  rox site
taactttaaataaggccggttatttaaagtta

SEQ ID NO: 42 - DNA, 23 bp, Artificial Sequence
  att site
tcagcttttttatactaagttgg

SEQ ID NO: 43 - DNA, 23 bp, Artificial Sequence
  att site
cctgcttttttatactaacttga

SEQ ID NO: 44 - DNA, 23 bp, Artificial Sequence
  att site
tgcgctaatttatacgaggctac

SEQ ID NO: 45 - DNA, 23 bp, Artificial Sequence
  att site
gcgtaatgtttataaatggcggc

SEQ ID NO: 46 - DNA, 23 bp, Artificial Sequence
  att site
cgcctttgttttcaaaaacctgc

SEQ ID NO: 47 - DNA, 23 bp, Artificial Sequence
  Artificial sequence
cgggcttttttctgtgtttcctg

SEQ ID NO: 48 - DNA, 23 bp, Artificial Sequence
  att site
ttggctattttaccacgactgtc